European Patent Application EP 4 183 804 A1, published May 24, 2023. Title: USE OF IL-36R ANTIBODIES FOR TREATMENT OF INFLAMMATORY BOWEL DISEASE. Applicant: BOECHER, WULF OTTO LAMAR, JANINE PADULA, STEVEN JOHN. The sequence listing filed with the application follows.

SEQUENCE LISTING (140 sequences)

SEQ ID NO: 1 - protein, 108 aa, Mus sp.
QIVLTQSPAIMSASLGERVTMTCTASSSVSSSYLHWYQKKPGSSPKLWVYSTSNLASGVPVRFSGSGSGTSYSLTISSMEAEDAATYYCHQHHRSPVTFGSGTKLEMK

SEQ ID NO: 2 - protein, 107 aa, Mus sp.
DIQMTQSPASQSASLGESVTFTCLASQTIGTWLAWYQQRPGKSPQLLIYAATSLADGVPSRFSGSGSGTQFSFNIRSLQAEDFASYYCQQVYTTPLTFGGGTKLEIK

SEQ ID NO: 3 - protein, 107 aa, Mus sp.
DIQMTQSPASQSASLGESVTFTCLASQTIGTWLGWYQQKPGKSPQLLIYRSTTLADGVPSRFSGSGSGTKFSFKISSLQAADFASYYCQQLYSAPYTFGGGTKLEIR

SEQ ID NO: 4 - protein, 112 aa, Mus sp.
DVLLTQTPLSLPVSLGDQASISCRSSQNIVHSNGNTYLQWYLQKPGQSPKLLIYKVSNRFSGVPDRFSGSGSGTDFTLKISRVEAEDLGVYYCFQGSHVPFTFGAGTKLELK

SEQ ID NO: 5 - protein, 107 aa, Artificial Sequence
  Description of Artificial Sequence: Synthetic polypeptide
DIQMTQTTSSLSASLGDRVTISCRASQDIYKYLNWYQQKPDGTLKLLIYYTSGLHSGVPSRFSGSGSGTDFSLTISNLEPEDIATYFCQQDSKFPWTFGGDTKLEIK

SEQ ID NO: 6 - protein, 108 aa, Mus sp.
QIVLTQSPAIMSASLGERVTMTCTASSSVSSSYFHWYQQKPGSSPKLWIYRTSNLASGVPGRFSGSGSGTSYSLTISSMEAEDAATYYCHQFHRSPLTFGAGTKLELK

SEQ ID NO: 7 - protein, 107 aa, Mus sp.
DIVMTQSQKFLSTSVGVRVSVTCKASQDVGTNVLWYQQKIGQSPKPLIYSASYRHSGVPDRFTGSGSGTDFTLIISNVQSEDLAEYFCQQYSRYPLTFGPGTKLELK

SEQ ID NO: 8 - protein, 107 aa, Mus sp.
DIVMTQSQKFLSTSVGVRVSVTCKASQDVGTNVLWYQQKIGQSPKALIYSASYRHSGVPDRFTGSGSGTDFTLIITNVQSEDLAEYFCQQYSRYPLTFGPGTKLELK

SEQ ID NO: 9 - protein, 107 aa, Mus sp.
DIVMTQSQKFMSATVGGRVNITCKASQNVGRAVAWYQQKPGQSPKLLTHSASNRYTGVPDRFTGSGSGTDFTLTITNMQSEDLADYFCQQYSSYPLTFGAGTKLDLK

SEQ ID NO: 10 - protein, 107 aa, Mus sp.
DIQMTQSPASQSASLGESVTFSCLASQTIGTWLGWYQQKPGKSPQLLIYRATSLADGVPSRFSGSGSGTNFSFKISSLQAEDLASYYCQQLYSGPYTFGGGTKLEIR

SEQ ID NO: 11 - protein, 119 aa, Mus sp.
QVQLQQSGTELLKPGASVKLSCKASGNTVTSYWMHWVKQRPGQGLEWIGEILPSTGRTNYNENFKGKAMLTVDKSSSTAYMQLSSLASEDSAVYYCTIVYFGNPWFAYWGQGTLVTVSA

SEQ ID NO: 12 - protein, 125 aa, Mus sp.
EVQLQQSGPELVKPGASVKLSCKASGYTFTDNYMNWVRQSHGKSLEWIGRVNPSNGDTKYNQNFKGKATLTVDKSLSTAYMQLNGLTSEDSAVYYCGRTKNFYSSYSYDDAMDYWGQGTSVTVSS

SEQ ID NO: 13 - protein, 124 aa, Mus sp.
EVQLQQSGAEFVRPGASVKFSCTASGFNIKDDYIHWVRQRPEQGLEWVGRIDPANGNTKYAPKFQDKATITADTSSNTAYLQLSSLTSEDTAVYYCAKSFPNNYYSYDDAFAYWGQGTLVTVSA

SEQ ID NO: 14 - protein, 118 aa, Mus sp.
QVQLKESGPVLVAPSQSLSITCTVSGFSLTKFGVHWIRQTPGKGLEWLGVIWAGGPTNYNSALMSRLTISKDISQSQVFLRIDSLQTDDTAMYYCAKQIYYSTLVDYWGQGTSVTVSS

SEQ ID NO: 15 - protein, 120 aa, Mus sp.
QVQLKESGPGLVAPSQSLFITCTVSGFSLSSYEINWVRQVPGKGLEWLGVIWTGITTNYNSALISRLSISKDNSKSLVFLKMNSLQTDDTAIYYCARGTGTGFYYAMDYWGQGTSVTVSS

SEQ ID NO: 16 - protein, 119 aa, Mus sp.
QVQLQQPGADFVRPGASMRLSCKASGYSFTSSWIHWVKQRPGQGLEWIGEINPGNVRTNYNENFRNKATLTVDKSSTTAYMQLRSLTSADSAVYYCTVVFYGEPYFPYWGQGTLVTVSA

SEQ ID NO: 17 - protein, 119 aa, Mus sp.
QVQLKESGPGLVAPSQSLSITCTVSGFSLTNYAVHWVRQFPGKGLEWLGVIWSDGSTDFNAPFKSRLSINKDNSKSQVFFKMNSLQIDDTAIYYCARKGGYSGSWFAYWGQGTLVTVSA

SEQ ID NO: 18 - protein, 119 aa, Mus sp.
QVQLKESGPGLVAPSQSLSITCTVSGFSLTNYAVHWVRQFPGKGLEWLGVIWSDGSTDYNAPFKSRLSINKDNSKSQVFFKMNSLQTDDTAIYYCARKGGYSGSWFAYWGQGTLVTVSA

SEQ ID NO: 19 - protein, 117 aa, Mus sp.
QVQLKESGPVLVAPSQSLSITCTVSGFSLTNYGVHWVRQPPGKGLEWLGVIWPVGSTNYNSALMSRLSIHKDNSKSQVFLRMNSLQTDDTAIYYCAKMDWDDFFDYWGQGTTLTVSS

SEQ ID NO: 20 - protein, 124 aa, Mus sp.
EVQLQQSGAELVRPGASVRLSCTASGFNIKDDYIHWVRQRPKQGLEWLGRIDPANGNTKYDPRFQDKATITADTSSNTAYLHLSSLTSEDTAVYYCAKSFPDNYYSYDDAFAYWGQGTLVTVSA

SEQ ID NO: 21 - protein, 12 aa, Mus sp.
TASSSVSSSYLH

SEQ ID NO: 22 - protein, 11 aa, Mus sp.
LASQTIGTWLA

SEQ ID NO: 23 - protein, 11 aa, Mus sp.
LASQTIGTWLG

SEQ ID NO: 24 - protein, 16 aa, Mus sp.
RSSQNIVHSNGNTYLQ

SEQ ID NO: 25 - protein, 11 aa, Mus sp.
RASQDIYKYLN

SEQ ID NO: 26 - protein, 12 aa, Mus sp.
TASSSVSSSYFH

SEQ ID NO: 27 - protein, 11 aa, Mus sp.
KASQDVGTNVL

SEQ ID NO: 28 - protein, 11 aa, Mus sp.
KASQNVGRAVA

SEQ ID NO: 29 - protein, 11 aa, Mus sp.
LASQTIGTWLG

SEQ ID NO: 30 - protein, 7 aa, Mus sp.
STSNLAS

SEQ ID NO: 31 - protein, 7 aa, Mus sp.
AATSLAD

SEQ ID NO: 32 - protein, 7 aa, Mus sp.
RSTTLAD

SEQ ID NO: 33 - protein, 7 aa, Mus sp.
KVSNRFS

SEQ ID NO: 34 - protein, 7 aa, Mus sp.
YTSGLHS

SEQ ID NO: 35 - protein, 7 aa, Mus sp.
RTSNLAS

SEQ ID NO: 36 - protein, 7 aa, Mus sp.
SASYRHS

SEQ ID NO: 37 - protein, 7 aa, Mus sp.
SASNRYT

SEQ ID NO: 38 - protein, 7 aa, Mus sp.
RATSLAD

SEQ ID NO: 39 - protein, 9 aa, Mus sp.
HQHHRSPVT

SEQ ID NO: 40 - protein, 9 aa, Artificial Sequence
  Description of Artificial Sequence: Synthetic peptide
QQVYTTPLT

SEQ ID NO: 41 - protein, 9 aa, Mus sp.
QQLYSAPYT

SEQ ID NO: 42 - protein, 9 aa, Mus sp.
FQGSHVPFT

SEQ ID NO: 43 - protein, 9 aa, Mus sp.
QQDSKFPWT

SEQ ID NO: 44 - protein, 9 aa, Mus sp.
HQFHRSPLT

SEQ ID NO: 45 - protein, 9 aa, Mus sp.
QQYSRYPLT

SEQ ID NO: 46 - protein, 9 aa, Mus sp.
QQYSSYPLT

SEQ ID NO: 47 - protein, 9 aa, Mus sp.
QQLYSGPYT

SEQ ID NO: 48 - protein, 10 aa, Mus sp.
GNTVTSYWMH

SEQ ID NO: 49 - protein, 10 aa, Mus sp.
GYTFTDNYMN

SEQ ID NO: 50 - protein, 10 aa, Mus sp.
GFNIKDDYIH

SEQ ID NO: 51 - protein, 10 aa, Mus sp.
GFSLTKFGVH

SEQ ID NO: 52 - protein, 10 aa, Mus sp.
GFSLSSYEIN

SEQ ID NO: 53 - protein, 10 aa, Mus sp.
GYSFTSSWIH

SEQ ID NO: 54 - protein, 10 aa, Mus sp.
GFSLTNYAVH

SEQ ID NO: 55 - protein, 10 aa, Mus sp.
GFSLTNYGVH

SEQ ID NO: 56 - protein, 10 aa, Mus sp.
GFNIKDDYIH

SEQ ID NO: 57 - protein, 17 aa, Mus sp.
EILPSTGRTNYNENFKG

SEQ ID NO: 58 - protein, 17 aa, Mus sp.
RVNPSNGDTKYNQNFKG

SEQ ID NO: 59 - protein, 17 aa, Mus sp.
RIDPANGNTKYAPKFQD

SEQ ID NO: 60 - protein, 16 aa, Mus sp.
VIWAGGPTNYNSALMS

SEQ ID NO: 61 - protein, 16 aa, Mus sp.
VIWTGITTNYNSALIS

SEQ ID NO: 62 - protein, 15 aa, Mus sp.
EINPGNVRTNYNENF

SEQ ID NO: 63 - protein, 16 aa, Mus sp.
VIWSDGSTDFNAPFKS

SEQ ID NO: 64 - protein, 16 aa, Mus sp.
VIWSDGSTDYNAPFKS

SEQ ID NO: 65 - protein, 16 aa, Mus sp.
VIWPVGSTNYNSALMS

SEQ ID NO: 66 - protein, 17 aa, Mus sp.
RIDPANGNTKYDPRFQD

SEQ ID NO: 67 - protein, 10 aa, Mus sp.
VYFGNPWFAY

SEQ ID NO: 68 - protein, 16 aa, Mus sp.
TKNFYSSYSYDDAMDY

SEQ ID NO: 69 - protein, 15 aa, Mus sp.
SFPNNYYSYDDAFAY

SEQ ID NO: 70 - protein, 10 aa, Mus sp.
QIYYSTLVDY

SEQ ID NO: 71 - protein, 12 aa, Mus sp.
GTGTGFYYAMDY

SEQ ID NO: 72 - protein, 10 aa, Mus sp.
VFYGEPYFPY

SEQ ID NO: 73 - protein, 11 aa, Mus sp.
KGGYSGSWFAY

SEQ ID NO: 74 - protein, 9 aa, Mus sp.
MDWDDFFDY

SEQ ID NO: 75 - protein, 15 aa, Mus sp.
SFPDNYYSYDDAFAY

SEQ ID NO: 76 - protein, 108 aa, Artificial Sequence
  Description of Artificial Sequence: Synthetic polypeptide
EIVLTQSPGTLSLSPGERATMSCTASSSVSSSYFHWYQQKPGQAPRLLIYRTSTLASGIPDRFSGSGSGTDFTLTISRLEPEDAATYYCHQFHRSPLTFGQGTKLEIK

SEQ ID NO: 77 - protein, 108 aa, Artificial Sequence
  Description of Artificial Sequence: Synthetic polypeptide
EIVLTQSPGTLSLSPGERATMSCTASSSVSSSYFHWYQQKPGQAPRLLIYRTSILASGVPDRFSGSGSGTDFTLTISRLEPEDFATYYCHQFHRSPLTFGQGTKLEIK

SEQ ID NO: 78 - protein, 108 aa, Artificial Sequence
  Description of Artificial Sequence: Synthetic polypeptide
EIVLTQSPGTLSLSPGERATMSCTASSSVSSSYFHWYQQKPGQAPRLWIYRTSRLASGVPDRFSGSGSGTDFTLTISRLEPEDAATYYCHQFHRSPLTFGQGTKLEIK

SEQ ID NO: 79 - protein, 108 aa, Artificial Sequence
  Description of Artificial Sequence: Synthetic polypeptide
EIVLTQSPGTLSLSPGERATMTCTASSSVSSSYFHWYQQKPGQAPRLLIYRTSRLASGVPDRFSGSGSGTDFTLTISRLEPEDFAVYYCHQFHRSPLTFGQGTKLEIK

SEQ ID NO: 80 - protein, 108 aa, Artificial Sequence [sequence omitted]

SEQ ID NO: 81 - protein, 108 aa, Artificial Sequence
  Description of Artificial Sequence: Synthetic polypeptide
QIVLTQSPGTLSLSPGERVTMSCTASSSVSSSYFHWYQQKPGQAPRLLIYRTSQLASGIPDRFSGSGSGTDFTLTISRLEPEDAATYYCHQFHRSPLTFGQGTKLEIK

SEQ ID NO: 82 - protein, 108 aa, Artificial Sequence
  Description of Artificial Sequence: Synthetic polypeptide
QIVLTQSPGTLSLSPGERATMTCTASSSVSSSYFHWYQQKPGQAPRLLIYRTSKLASGVPDRFSGSGSGTDFTLTISRLEPEDFATYYCHQFHRSPLTFGQGTKLEIK

SEQ ID NO: 83 - protein, 108 aa, Artificial Sequence
  Description of Artificial Sequence: Synthetic polypeptide
EIVLTQSPGTLSLSPGERATMSCTASSSVSSSYFHWYQQKPGQAPRLLIYRTSHLASGIPGRFSGSGSGTDFTLTISRLEPEDAAVYYCHQFHRSPLTFGQGTKLEIK

SEQ ID NO: 84 - protein, 107 aa, Artificial Sequence
  Description of Artificial Sequence: Synthetic polypeptide
EIVMTQSPATLSVSPGVRATLSCKASQDVGTNVLWYQQKPGQAPRPLIYSASYRHSGIPDRFSGSGSGTEFTLTISSLQSEDFAEYFCQQYSRYPLTFGQGTKLEIK

SEQ ID NO: 85 - protein, 107 aa, Artificial Sequence
  Description of Artificial Sequence: Synthetic polypeptide
EIVMTQSPATLSVSPGVRATLSCKASQDVGTNVLWYQQKPGQAPRPLIYSASYRHSGIPDRFSGSGSGTEFTLTISSLQSEDFAVYYCQQYSRYPLTFGQGTKLEIK

SEQ ID NO: 86 - protein, 107 aa, Artificial Sequence
  Description of Artificial Sequence: Synthetic polypeptide
EIVMTQSPATLSVSPGVRATLSCKASQDVGTNVLWYQQKPGQAPRPLIYSASYRHSGIPARFSGSGSGTEFTLTISSLQSEDFAEYYCQQYSRYPLTFGQGTKLEIK

SEQ ID NO: 87 - protein, 119 aa, Artificial Sequence
  Description of Artificial Sequence: Synthetic polypeptide
QVQLVQSGAEVKKPGASVKVSCKASGYSFTSSWIHWVRQAPGQGLEWIGEINPGNVRTNYNENFRNKATMTVDTSISTAYMELSRLRSDDTAVYYCAVVFYGEPYFPYWGQGTLVTVSS

SEQ ID NO: 88 - protein, 119 aa, Artificial Sequence
  Description of Artificial Sequence: Synthetic polypeptide
QVQLVQSGAEVKKPGASVKVSCKASGYSFTSSWIHWVRQRPGQGLEWIGEINPGNVRTNYNENFRNRVTMTVDTSISTAYMELSRLRSDDTAVYYCTVVFYGEPYFPYWGQGTLVTVSS

SEQ ID NO: 89 - protein, 119 aa, Artificial Sequence [sequence omitted]

SEQ ID NO: 90 - protein, 119 aa, Artificial Sequence
  Description of Artificial Sequence: Synthetic polypeptide
QVQLVQSGAEVKKPGASVKVSCKASGYSFTSSWIHWVRQRPGQGLEWMGEINPGNVRTNYNENFRNRATLTRDTSISTAYMELSRLRSDDTAVYYCAVVFYGEPYFPYWGQGTLVTVSS

SEQ ID NO: 91 - protein, 119 aa, Artificial Sequence
  Description of Artificial Sequence: Synthetic polypeptide
QVQLVQSGAEVKKPGASVKVSCKASGYSFTSSWIHWVRQRPGQGLEWMGEILPGVVRTNYNENFRNKVTMTVDTSISTAYMELSRLRSDDTAVYYCTVVFYGEPYFPYWGQGTLVTVSS

SEQ ID NO: 92 - protein, 119 aa, Artificial Sequence
  Description of Artificial Sequence: Synthetic polypeptide
QVQLVQSGAEVKKPGASVKVSCKASGYSFTSSWIHWVRQRPGQGLEWIGEINPGAVRTNYNENFRNRVTMTVDTSISTAYMELSRLRSDDTAVYYCTVVFYGEPYFPYWGQGTLVTVSS

SEQ ID NO: 93 - protein, 119 aa, Artificial Sequence
  Description of Artificial Sequence: Synthetic polypeptide
QVQLVQSGAEVKKPGASVKVSCKASGYSFTSSWIHWVRQAPGQGLEWIGEINPGLVRTNYNENFRNKVTMTVDTSISTAYMELSRLRSDDTAVYYCAVVFYGEPYFPYWGQGTLVTVSS

SEQ ID NO: 94 - protein, 119 aa, Artificial Sequence
  Description of Artificial Sequence: Synthetic polypeptide
QVQLVQSGAEVKKPGASVKVSCKASGYSFTSSWIHWVRQAPGQGLEWIGEINPGAVRTNYNENFRNKVTMTVDTSISTAYMELSRLRSDDTAVYYCAVVFYGEPYFPYWGQGTLVTVSS

SEQ ID NO: 95 - protein, 119 aa, Artificial Sequence
  Description of Artificial Sequence: Synthetic polypeptide
QVQLVQSGAEVKKPGASVKVSCKASGYSFTSSWIHWVRQAPGQGLEWIGEINPGSVRTNYNENFRNKATMTVDTSISTAYMELSRLRSDDTAVYYCAVVFYGEPYFPYWGQGTLVTVSS

SEQ ID NO: 96 - protein, 119 aa, Artificial Sequence
  Description of Artificial Sequence: Synthetic polypeptide
QVQLQESGPGLVKPSETLSITCTVSGFSLTDYAVHWIRQPPGKGLEWIGVIWSDGSTDYNAPFKSRVTINKDTSKSQVSFKMSSVQAADTAVYYCARKGGYSGSWFAYWGQGTLVTVSS

SEQ ID NO: 97 - protein, 119 aa, Artificial Sequence
  Description of Artificial Sequence: Synthetic polypeptide
QVQLQESGPGLVKPSETLSITCTVSGFSLTDYAVHWIRQPPGKGLEWIGVIWSDGSTDYNAPFKSRVTISKDTSKNQVSLKMNSLTTDDTAVYYCARKGGYSGSWFAYWGQGTLVTVSS

SEQ ID NO: 98 - protein, 119 aa, Artificial Sequence
  Description of Artificial Sequence: Synthetic polypeptide
QVQLQESGPGLVKPSETLSITCTVSGFSLTDYAVHWIRQPPGKGLEWIGVIWSDGSTDYNAPFKSRVTISKDNSKSQVSLKMNSVTVADTAVYYCARKGGYSGSWFAYWGQGTLVTVSS

SEQ ID NO: 99 - protein, 119 aa, Artificial Sequence
  Description of Artificial Sequence: Synthetic polypeptide
QVQLQESGPGLVKPSETLSITCTVSGFSLTDYAVHWVRQPPGKGLEWIGVIWSDGSTDYNAPFKSRVTISKDTSKNQVSFKLSSVTVDDTAVYYCARKGGYSGSWFAYWGQGTLVTVSS

SEQ ID NO: 100 - protein, 119 aa, Artificial Sequence
  Description of Artificial Sequence: Synthetic polypeptide
QVQLQESGPGLVAPSETLSLTCTVSGFSLTDYAVHWIRQFPGKGLEWIGVIWSDGSTDFNAPFKSRVTISKDTSKNQVSFKLSSVTTDDTAVYYCARKGGYSGSWFAYWGQGTLVTVSS

SEQ ID NO: 101 - protein, 119 aa, Artificial Sequence
  Description of Artificial Sequence: Synthetic polypeptide
QVQLQESGPGLVKPSETLSITCTVSGFSLTDYAVHWIRQPPGKGLEWIGVIWSDGSTDYNAPFKSRVTISKDNSKSQVSFKMSSVTADDTAVYYCARKGGYSGSWFAYWGQGTLVTVSS

SEQ ID NO: 102 - protein, 7 aa, Mus sp.
RTSTLAS

SEQ ID NO: 103 - protein, 7 aa, Mus sp.
RTSILAS

SEQ ID NO: 104 - protein, 7 aa, Mus sp.
RTSRLAS

SEQ ID NO: 105 - protein, 7 aa, Mus sp.
RTSQLAS

SEQ ID NO: 106 - protein, 7 aa, Mus sp.
RTSKLAS

SEQ ID NO: 107 - protein, 10 aa, Mus sp.
GFSLTDYAVH

SEQ ID NO: 108 - protein, 15 aa, Mus sp.
EILPGVVRTNYNENF

SEQ ID NO: 109 - protein, 15 aa, Mus sp.
EINPGAVRTNYNENF

SEQ ID NO: 110 - protein, 15 aa, Mus sp.
EINPGLVRTNYNENF

SEQ ID NO: 111 - protein, 15 aa, Mus sp.
EINPGSVRTNYNENF

SEQ ID NO: 112 - protein, 330 aa, Artificial Sequence
  Description of Artificial Sequence: Synthetic polypeptide
ASTKGPSVFPLAPSSKSTSGGTAALGCLVKDYFPEPVTVSWNSGALTSGVHTFPAVLQSSGLYSLSSVVTVPSSSLGTQTYICNVNHKPSNTKVDKRVEPKSCDKTHTCPPCPAPEAAGGPSVFLFPPKPKDTLMISRTPEVTCVVVDVSHEDPEVKFNWYVDGVEVHNAKTKPREEQYNSTYRVVSVLTVLHQDWLNGKEYKCKVSNKALPAPIEKTISKAKGQPREPQVYTLPPSREEMTKNQVSLTCLVKGFYPSDIAVEWESNGQPENNYKTTPPVLDSDGSFFLYSKLTVDKSRWQQGNVFSCSVMHEALHNHYTQKSLSLSPGK

SEQ ID NO: 113 - protein, 107 aa, Artificial Sequence [sequence omitted]

SEQ ID NO: 114 - protein, 215 aa, Artificial Sequence
  Description of Artificial Sequence: Synthetic polypeptide
EIVLTQSPGTLSLSPGERATMSCTASSSVSSSYFHWYQQKPGQAPRLLIYRTSTLASGIPDRFSGSGSGTDFTLTISRLEPEDAATYYCHQFHRSPLTFGQGTKLEIKRTVAAPSVFIFPPSDEQLKSGTASVVCLLNNFYPREAKVQWKVDNALQSGNSQESVTEQDSKDSTYSLSSTLTLSKADYEKHKVYACEVTHQGLSSPVTKSFNRGEC

SEQ ID NO: 115 - protein, 215 aa, Artificial Sequence
  Description of Artificial Sequence: Synthetic polypeptide
EIVLTQSPGTLSLSPGERATMSCTASSSVSSSYFHWYQQKPGQAPRLLIYRTSILASGVPDRFSGSGSGTDFTLTISRLEPEDFATYYCHQFHRSPLTFGQGTKLEIKRTVAAPSVFIFPPSDEQLKSGTASVVCLLNNFYPREAKVQWKVDNALQSGNSQESVTEQDSKDSTYSLSSTLTLSKADYEKHKVYACEVTHQGLSSPVTKSFNRGEC

SEQ ID NO: 116 - protein, 215 aa, Artificial Sequence
  Description of Artificial Sequence: Synthetic polypeptide
EIVLTQSPGTLSLSPGERATMSCTASSSVSSSYFHWYQQKPGQAPRLWIYRTSRLASGVPDRFSGSGSGTDFTLTISRLEPEDAATYYCHQFHRSPLTFGQGTKLEIKRTVAAPSVFIFPPSDEQLKSGTASVVCLLNNFYPREAKVQWKVDNALQSGNSQESVTEQDSKDSTYSLSSTLTLSKADYEKHKVYACEVTHQGLSSPVTKSFNRGEC

SEQ ID NO: 117 - protein, 215 aa, Artificial Sequence
  Description of Artificial Sequence: Synthetic polypeptide
EIVLTQSPGTLSLSPGERATMTCTASSSVSSSYFHWYQQKPGQAPRLLIYRTSRLASGVPDRFSGSGSGTDFTLTISRLEPEDFAVYYCHQFHRSPLTFGQGTKLEIKRTVAAPSVFIFPPSDEQLKSGTASVVCLLNNFYPREAKVQWKVDNALQSGNSQESVTEQDSKDSTYSLSSTLTLSKADYEKHKVYACEVTHQGLSSPVTKSFNRGEC

SEQ ID NO: 118 - protein, 215 aa, Artificial Sequence
  Description of Artificial Sequence: Synthetic polypeptide
QIVLTQSPGTLSLSPGERATMTCTASSSVSSSYFHWYQQKPGQAPRLWIYRTSRLASGVPDRFSGSGSGTDFTLTISRLEPEDAATYYCHQFHRSPLTFGAGTKLEIKRTVAAPSVFIFPPSDEQLKSGTASVVCLLNNFYPREAKVQWKVDNALQSGNSQESVTEQDSKDSTYSLSSTLTLSKADYEKHKVYACEVTHQGLSSPVTKSFNRGEC

SEQ ID NO: 119 - protein, 215 aa, Artificial Sequence
  Description of Artificial Sequence: Synthetic polypeptide
QIVLTQSPGTLSLSPGERVTMSCTASSSVSSSYFHWYQQKPGQAPRLLIYRTSQLASGIPDRFSGSGSGTDFTLTISRLEPEDAATYYCHQFHRSPLTFGQGTKLEIKRTVAAPSVFIFPPSDEQLKSGTASVVCLLNNFYPREAKVQWKVDNALQSGNSQESVTEQDSKDSTYSLSSTLTLSKADYEKHKVYACEVTHQGLSSPVTKSFNRGEC

SEQ ID NO: 120 - protein, 215 aa, Artificial Sequence
  Description of Artificial Sequence: Synthetic polypeptide
QIVLTQSPGTLSLSPGERATMTCTASSSVSSSYFHWYQQKPGQAPRLLIYRTSKLASGVPDRFSGSGSGTDFTLTISRLEPEDFATYYCHQFHRSPLTFGQGTKLEIKRTVAAPSVFIFPPSDEQLKSGTASVVCLLNNFYPREAKVQWKVDNALQSGNSQESVTEQDSKDSTYSLSSTLTLSKADYEKHKVYACEVTHQGLSSPVTKSFNRGEC

SEQ ID NO: 121 - protein, 215 aa, Artificial Sequence
  Description of Artificial Sequence: Synthetic polypeptide
EIVLTQSPGTLSLSPGERATMSCTASSSVSSSYFHWYQQKPGQAPRLLIYRTSHLASGIPGRFSGSGSGTDFTLTISRLEPEDAAVYYCHQFHRSPLTFGQGTKLEIKRTVAAPSVFIFPPSDEQLKSGTASVVCLLNNFYPREAKVQWKVDNALQSGNSQESVTEQDSKDSTYSLSSTLTLSKADYEKHKVYACEVTHQGLSSPVTKSFNRGEC

SEQ ID NO: 122 - protein, 214 aa, Artificial Sequence
  Description of Artificial Sequence: Synthetic polypeptide
EIVMTQSPATLSVSPGVRATLSCKASQDVGTNVLWYQQKPGQAPRPLIYSASYRHSGIPDRFSGSGSGTEFTLTISSLQSEDFAEYFCQQYSRYPLTFGQGTKLEIKRTVAAPSVFIFPPSDEQLKSGTASVVCLLNNFYPREAKVQWKVDNALQSGNSQESVTEQDSKDSTYSLSSTLTLSKADYEKHKVYACEVTHQGLSSPVTKSFNRGEC

SEQ ID NO: 123 - protein, 214 aa, Artificial Sequence
  Description of Artificial Sequence: Synthetic polypeptide
EIVMTQSPATLSVSPGVRATLSCKASQDVGTNVLWYQQKPGQAPRPLIYSASYRHSGIPDRFSGSGSGTEFTLTISSLQSEDFAVYYCQQYSRYPLTFGQGTKLEIKRTVAAPSVFIFPPSDEQLKSGTASVVCLLNNFYPREAKVQWKVDNALQSGNSQESVTEQDSKDSTYSLSSTLTLSKADYEKHKVYACEVTHQGLSSPVTKSFNRGEC

SEQ ID NO: 124 - protein, 214 aa, Artificial Sequence
  Description of Artificial Sequence: Synthetic polypeptide
EIVMTQSPATLSVSPGVRATLSCKASQDVGTNVLWYQQKPGQAPRPLIYSASYRHSGIPARFSGSGSGTEFTLTISSLQSEDFAEYYCQQYSRYPLTFGQGTKLEIKRTVAAPSVFIFPPSDEQLKSGTASVVCLLNNFYPREAKVQWKVDNALQSGNSQESVTEQDSKDSTYSLSSTLTLSKADYEKHKVYACEVTHQGLSSPVTKSFNRGEC

SEQ ID NO: 125 - protein, 449 aa, Artificial Sequence
  Description of Artificial Sequence: Synthetic polypeptide
QVQLVQSGAEVKKPGASVKVSCKASGYSFTSSWIHWVRQAPGQGLEWIGEINPGNVRTNYNENFRNKATMTVDTSISTAYMELSRLRSDDTAVYYCAVVFYGEPYFPYWGQGTLVTVSSASTKGPSVFPLAPSSKSTSGGTAALGCLVKDYFPEPVTVSWNSGALTSGVHTFPAVLQSSGLYSLSSVVTVPSSSLGTQTYICNVNHKPSNTKVDKRVEPKSCDKTHTCPPCPAPEAAGGPSVFLFPPKPKDTLMISRTPEVTCVVVDVSHEDPEVKFNWYVDGVEVHNAKTKPREEQYNSTYRVVSVLTVLHQDWLNGKEYKCKVSNKALPAPIEKTISKAKGQPREPQVYTLPPSREEMTKNQVSLTCLVKGFYPSDIAVEWESNGQPENNYKTTPPVLDSDGSFFLYSKLTVDKSRWQQGNVFSCSVMHEALHNHYTQKSLSLSPGK

SEQ ID NO: 126 - protein, 449 aa, Artificial Sequence
  Description of Artificial Sequence: Synthetic polypeptide
QVQLVQSGAEVKKPGASVKVSCKASGYSFTSSWIHWVRQRPGQGLEWIGEINPGNVRTNYNENFRNRVTMTVDTSISTAYMELSRLRSDDTAVYYCTVVFYGEPYFPYWGQGTLVTVSSASTKGPSVFPLAPSSKSTSGGTAALGCLVKDYFPEPVTVSWNSGALTSGVHTFPAVLQSSGLYSLSSVVTVPSSSLGTQTYICNVNHKPSNTKVDKRVEPKSCDKTHTCPPCPAPEAAGGPSVFLFPPKPKDTLMISRTPEVTCVVVDVSHEDPEVKFNWYVDGVEVHNAKTKPREEQYNSTYRVVSVLTVLHQDWLNGKEYKCKVSNKALPAPIEKTISKAKGQPREPQVYTLPPSREEMTKNQVSLTCLVKGFYPSDIAVEWESNGQPENNYKTTPPVLDSDGSFFLYSKLTVDKSRWQQGNVFSCSVMHEALHNHYTQKSLSLSPGK

SEQ ID NO: 127 - protein, 449 aa, Artificial Sequence
  Description of Artificial Sequence: Synthetic polypeptide
QVQLVQSGAEVKKPGASVKVSCKASGYSFTSSWIHWVKQAPGQGLEWMGEINPGNVRTNYNENFRNKVTMTVDTSISTAYMELSRLRSDDTAVYYCTVVFYGEPYFPYWGQGTLVTVSSASTKGPSVFPLAPSSKSTSGGTAALGCLVKDYFPEPVTVSWNSGALTSGVHTFPAVLQSSGLYSLSSVVTVPSSSLGTQTYICNVNHKPSNTKVDKRVEPKSCDKTHTCPPCPAPEAAGGPSVFLFPPKPKDTLMISRTPEVTCVVVDVSHEDPEVKFNWYVDGVEVHNAKTKPREEQYNSTYRVVSVLTVLHQDWLNGKEYKCKVSNKALPAPIEKTISKAKGQPREPQVYTLPPSREEMTKNQVSLTCLVKGFYPSDIAVEWESNGQPENNYKTTPPVLDSDGSFFLYSKLTVDKSRWQQGNVFSCSVMHEALHNHYTQKSLSLSPGK

SEQ ID NO: 128 - protein, 449 aa, Artificial Sequence
  Description of Artificial Sequence: Synthetic polypeptide
QVQLVQSGAEVKKPGASVKVSCKASGYSFTSSWIHWVRQRPGQGLEWMGEINPGNVRTNYNENFRNRATLTRDTSISTAYMELSRLRSDDTAVYYCAVVFYGEPYFPYWGQGTLVTVSSASTKGPSVFPLAPSSKSTSGGTAALGCLVKDYFPEPVTVSWNSGALTSGVHTFPAVLQSSGLYSLSSVVTVPSSSLGTQTYICNVNHKPSNTKVDKRVEPKSCDKTHTCPPCPAPEAAGGPSVFLFPPKPKDTLMISRTPEVTCVVVDVSHEDPEVKFNWYVDGVEVHNAKTKPREEQYNSTYRVVSVLTVLHQDWLNGKEYKCKVSNKALPAPIEKTISKAKGQPREPQVYTLPPSREEMTKNQVSLTCLVKGFYPSDIAVEWESNGQPENNYKTTPPVLDSDGSFFLYSKLTVDKSRWQQGNVFSCSVMHEALHNHYTQKSLSLSPGK

SEQ ID NO: 129 - protein, 449 aa, Artificial Sequence
  Description of Artificial Sequence: Synthetic polypeptide
QVQLVQSGAEVKKPGASVKVSCKASGYSFTSSWIHWVRQRPGQGLEWMGEILPGVVRTNYNENFRNKVTMTVDTSISTAYMELSRLRSDDTAVYYCTVVFYGEPYFPYWGQGTLVTVSSASTKGPSVFPLAPSSKSTSGGTAALGCLVKDYFPEPVTVSWNSGALTSGVHTFPAVLQSSGLYSLSSVVTVPSSSLGTQTYICNVNHKPSNTKVDKRVEPKSCDKTHTCPPCPAPEAAGGPSVFLFPPKPKDTLMISRTPEVTCVVVDVSHEDPEVKFNWYVDGVEVHNAKTKPREEQYNSTYRVVSVLTVLHQDWLNGKEYKCKVSNKALPAPIEKTISKAKGQPREPQVYTLPPSREEMTKNQVSLTCLVKGFYPSDIAVEWESNGQPENNYKTTPPVLDSDGSFFLYSKLTVDKSRWQQGNVFSCSVMHEALHNHYTQKSLSLSPGK

SEQ ID NO: 130 - protein, 449 aa, Artificial Sequence
  Description of Artificial Sequence: Synthetic polypeptide
QVQLVQSGAEVKKPGASVKVSCKASGYSFTSSWIHWVRQRPGQGLEWIGEINPGAVRTNYNENFRNRVTMTVDTSISTAYMELSRLRSDDTAVYYCTVVFYGEPYFPYWGQGTLVTVSSASTKGPSVFPLAPSSKSTSGGTAALGCLVKDYFPEPVTVSWNSGALTSGVHTFPAVLQSSGLYSLSSVVTVPSSSLGTQTYICNVNHKPSNTKVDKRVEPKSCDKTHTCPPCPAPEAAGGPSVFLFPPKPKDTLMISRTPEVTCVVVDVSHEDPEVKFNWYVDGVEVHNAKTKPREEQYNSTYRVVSVLTVLHQDWLNGKEYKCKVSNKALPAPIEKTISKAKGQPREPQVYTLPPSREEMTKNQVSLTCLVKGFYPSDIAVEWESNGQPENNYKTTPPVLDSDGSFFLYSKLTVDKSRWQQGNVFSCSVMHEALHNHYTQKSLSLSPGK

SEQ ID NO: 131 - protein, 449 aa, Artificial Sequence
  Description of Artificial Sequence: Synthetic polypeptide
QVQLVQSGAEVKKPGASVKVSCKASGYSFTSSWIHWVRQAPGQGLEWIGEINPGLVRTNYNENFRNKVTMTVDTSISTAYMELSRLRSDDTAVYYCAVVFYGEPYFPYWGQGTLVTVSSASTKGPSVFPLAPSSKSTSGGTAALGCLVKDYFPEPVTVSWNSGALTSGVHTFPAVLQSSGLYSLSSVVTVPSSSLGTQTYICNVNHKPSNTKVDKRVEPKSCDKTHTCPPCPAPEAAGGPSVFLFPPKPKDTLMISRTPEVTCVVVDVSHEDPEVKFNWYVDGVEVHNAKTKPREEQYNSTYRVVSVLTVLHQDWLNGKEYKCKVSNKALPAPIEKTISKAKGQPREPQVYTLPPSREEMTKNQVSLTCLVKGFYPSDIAVEWESNGQPENNYKTTPPVLDSDGSFFLYSKLTVDKSRWQQGNVFSCSVMHEALHNHYTQKSLSLSPGK

SEQ ID NO: 132 - protein, 449 aa, Artificial Sequence
  Description of Artificial Sequence: Synthetic polypeptide
QVQLVQSGAEVKKPGASVKVSCKASGYSFTSSWIHWVRQAPGQGLEWIGEINPGAVRTNYNENFRNKVTMTVDTSISTAYMELSRLRSDDTAVYYCAVVFYGEPYFPYWGQGTLVTVSSASTKGPSVFPLAPSSKSTSGGTAALGCLVKDYFPEPVTVSWNSGALTSGVHTFPAVLQSSGLYSLSSVVTVPSSSLGTQTYICNVNHKPSNTKVDKRVEPKSCDKTHTCPPCPAPEAAGGPSVFLFPPKPKDTLMISRTPEVTCVVVDVSHEDPEVKFNWYVDGVEVHNAKTKPREEQYNSTYRVVSVLTVLHQDWLNGKEYKCKVSNKALPAPIEKTISKAKGQPREPQVYTLPPSREEMTKNQVSLTCLVKGFYPSDIAVEWESNGQPENNYKTTPPVLDSDGSFFLYSKLTVDKSRWQQGNVFSCSVMHEALHNHYTQKSLSLSPGK

SEQ ID NO: 133 - protein, 449 aa, Artificial Sequence
  Description of Artificial Sequence: Synthetic polypeptide
QVQLVQSGAEVKKPGASVKVSCKASGYSFTSSWIHWVRQAPGQGLEWIGEINPGSVRTNYNENFRNKATMTVDTSISTAYMELSRLRSDDTAVYYCAVVFYGEPYFPYWGQGTLVTVSSASTKGPSVFPLAPSSKSTSGGTAALGCLVKDYFPEPVTVSWNSGALTSGVHTFPAVLQSSGLYSLSSVVTVPSSSLGTQTYICNVNHKPSNTKVDKRVEPKSCDKTHTCPPCPAPEAAGGPSVFLFPPKPKDTLMISRTPEVTCVVVDVSHEDPEVKFNWYVDGVEVHNAKTKPREEQYNSTYRVVSVLTVLHQDWLNGKEYKCKVSNKALPAPIEKTISKAKGQPREPQVYTLPPSREEMTKNQVSLTCLVKGFYPSDIAVEWESNGQPENNYKTTPPVLDSDGSFFLYSKLTVDKSRWQQGNVFSCSVMHEALHNHYTQKSLSLSPGK

SEQ ID NO: 134 - protein, 449 aa, Artificial Sequence
  Description of Artificial Sequence: Synthetic polypeptide
QVQLQESGPGLVKPSETLSITCTVSGFSLTDYAVHWIRQPPGKGLEWIGVIWSDGSTDYNAPFKSRVTINKDTSKSQVSFKMSSVQAADTAVYYCARKGGYSGSWFAYWGQGTLVTVSSASTKGPSVFPLAPSSKSTSGGTAALGCLVKDYFPEPVTVSWNSGALTSGVHTFPAVLQSSGLYSLSSVVTVPSSSLGTQTYICNVNHKPSNTKVDKRVEPKSCDKTHTCPPCPAPEAAGGPSVFLFPPKPKDTLMISRTPEVTCVVVDVSHEDPEVKFNWYVDGVEVHNAKTKPREEQYNSTYRVVSVLTVLHQDWLNGKEYKCKVSNKALPAPIEKTISKAKGQPREPQVYTLPPSREEMTKNQVSLTCLVKGFYPSDIAVEWESNGQPENNYKTTPPVLDSDGSFFLYSKLTVDKSRWQQGNVFSCSVMHEALHNHYTQKSLSLSPGK

SEQ ID NO: 135 - protein, 449 aa, Artificial Sequence
  Description of Artificial Sequence: Synthetic polypeptide
QVQLQESGPGLVKPSETLSITCTVSGFSLTDYAVHWIRQPPGKGLEWIGVIWSDGSTDYNAPFKSRVTISKDTSKNQVSLKMNSLTTDDTAVYYCARKGGYSGSWFAYWGQGTLVTVSSASTKGPSVFPLAPSSKSTSGGTAALGCLVKDYFPEPVTVSWNSGALTSGVHTFPAVLQSSGLYSLSSVVTVPSSSLGTQTYICNVNHKPSNTKVDKRVEPKSCDKTHTCPPCPAPEAAGGPSVFLFPPKPKDTLMISRTPEVTCVVVDVSHEDPEVKFNWYVDGVEVHNAKTKPREEQYNSTYRVVSVLTVLHQDWLNGKEYKCKVSNKALPAPIEKTISKAKGQPREPQVYTLPPSREEMTKNQVSLTCLVKGFYPSDIAVEWESNGQPENNYKTTPPVLDSDGSFFLYSKLTVDKSRWQQGNVFSCSVMHEALHNHYTQKSLSLSPGK

SEQ ID NO: 136 - protein, 449 aa, Artificial Sequence
  Description of Artificial Sequence: Synthetic polypeptide
QVQLQESGPGLVKPSETLSITCTVSGFSLTDYAVHWIRQPPGKGLEWIGVIWSDGSTDYNAPFKSRVTISKDNSKSQVSLKMNSVTVADTAVYYCARKGGYSGSWFAYWGQGTLVTVSSASTKGPSVFPLAPSSKSTSGGTAALGCLVKDYFPEPVTVSWNSGALTSGVHTFPAVLQSSGLYSLSSVVTVPSSSLGTQTYICNVNHKPSNTKVDKRVEPKSCDKTHTCPPCPAPEAAGGPSVFLFPPKPKDTLMISRTPEVTCVVVDVSHEDPEVKFNWYVDGVEVHNAKTKPREEQYNSTYRVVSVLTVLHQDWLNGKEYKCKVSNKALPAPIEKTISKAKGQPREPQVYTLPPSREEMTKNQVSLTCLVKGFYPSDIAVEWESNGQPENNYKTTPPVLDSDGSFFLYSKLTVDKSRWQQGNVFSCSVMHEALHNHYTQKSLSLSPGK

SEQ ID NO: 137 - protein, 449 aa, Artificial Sequence
  Description of Artificial Sequence: Synthetic polypeptide
QVQLQESGPGLVKPSETLSITCTVSGFSLTDYAVHWVRQPPGKGLEWIGVIWSDGSTDYNAPFKSRVTISKDTSKNQVSFKLSSVTVDDTAVYYCARKGGYSGSWFAYWGQGTLVTVSSASTKGPSVFPLAPSSKSTSGGTAALGCLVKDYFPEPVTVSWNSGALTSGVHTFPAVLQSSGLYSLSSVVTVPSSSLGTQTYICNVNHKPSNTKVDKRVEPKSCDKTHTCPPCPAPEAAGGPSVFLFPPKPKDTLMISRTPEVTCVVVDVSHEDPEVKFNWYVDGVEVHNAKTKPREEQYNSTYRVVSVLTVLHQDWLNGKEYKCKVSNKALPAPIEKTISKAKGQPREPQVYTLPPSREEMTKNQVSLTCLVKGFYPSDIAVEWESNGQPENNYKTTPPVLDSDGSFFLYSKLTVDKSRWQQGNVFSCSVMHEALHNHYTQKSLSLSPGK

SEQ ID NO: 138 - protein, 449 aa, Artificial Sequence
  Description of Artificial Sequence: Synthetic polypeptide
QVQLQESGPGLVAPSETLSLTCTVSGFSLTDYAVHWIRQFPGKGLEWIGVIWSDGSTDFNAPFKSRVTISKDTSKNQVSFKLSSVTTDDTAVYYCARKGGYSGSWFAYWGQGTLVTVSSASTKGPSVFPLAPSSKSTSGGTAALGCLVKDYFPEPVTVSWNSGALTSGVHTFPAVLQSSGLYSLSSVVTVPSSSLGTQTYICNVNHKPSNTKVDKRVEPKSCDKTHTCPPCPAPEAAGGPSVFLFPPKPKDTLMISRTPEVTCVVVDVSHEDPEVKFNWYVDGVEVHNAKTKPREEQYNSTYRVVSVLTVLHQDWLNGKEYKCKVSNKALPAPIEKTISKAKGQPREPQVYTLPPSREEMTKNQVSLTCLVKGFYPSDIAVEWESNGQPENNYKTTPPVLDSDGSFFLYSKLTVDKSRWQQGNVFSCSVMHEALHNHYTQKSLSLSPGK

SEQ ID NO: 139 - protein, 449 aa, Artificial Sequence
  Description of Artificial Sequence: Synthetic polypeptide
QVQLQESGPGLVKPSETLSITCTVSGFSLTDYAVHWIRQPPGKGLEWIGVIWSDGSTDYNAPFKSRVTISKDNSKSQVSFKMSSVTADDTAVYYCARKGGYSGSWFAYWGQGTLVTVSSASTKGPSVFPLAPSSKSTSGGTAALGCLVKDYFPEPVTVSWNSGALTSGVHTFPAVLQSSGLYSLSSVVTVPSSSLGTQTYICNVNHKPSNTKVDKRVEPKSCDKTHTCPPCPAPEAAGGPSVFLFPPKPKDTLMISRTPEVTCVVVDVSHEDPEVKFNWYVDGVEVHNAKTKPREEQYNSTYRVVSVLTVLHQDWLNGKEYKCKVSNKALPAPIEKTISKAKGQPREPQVYTLPPSREEMTKNQVSLTCLVKGFYPSDIAVEWESNGQPENNYKTTPPVLDSDGSFFLYSKLTVDKSRWQQGNVFSCSVMHEALHNHYTQKSLSLSPGK

SEQ ID NO: 140 - protein, 7 aa, Mus sp.
RTSHLAS